European Patent Application EP 4 541 879 A1, published April 23, 2025. Title: Vessel for single-cell analysis and a method using the same. Applicant: Hitachi, Ltd. The sequence listing filed with the application follows.

SEQUENCE LISTING (96 sequences)

SEQ ID NO: 1 - DNA, 65 bp, synthetic construct
  misc_feature 1..65: note = synthetic oligonucleotide
  misc_feature 39..45: note = n is a, c, g, or t
  misc_feature 65: note = n is a, c, g, or t
  source 1..65: mol_type = other DNA
ccatctcatccctgcgtgtctccgactcagtcgcgtacnnnnnnnttttttttttttttttttvn

SEQ ID NO: 2 - DNA, 21 bp, synthetic construct
  misc_feature 1..21: note = synthetic oligonucleotide
  source 1..21: mol_type = other DNA
ccatctcatccctgcgtgtct

SEQ ID NO: 3 - DNA, 58 bp, synthetic construct
  misc_feature 1..58: note = synthetic oligonucleotide
  source 1..58: mol_type = other DNA
aatgatacggcgaccaccgagatctacactctttccctacacgacgctcttccgatct

SEQ ID NO: 4 - DNA, 58 bp, synthetic construct
  misc_feature 1..58: note = synthetic oligonucleotide
  source 1..58: mol_type = other DNA
caagcagaagacggcatacgagatgtgactggagttcagacgtgtgctcttccgatct

SEQ ID NO: 5 - DNA, 87 bp, synthetic construct
  misc_feature 1..87: note = synthetic oligonucleotide
  source 1..87: mol_type = other DNA
aatgatacggcgaccaccgagatctacactctttccctacacgacgctcttccgatcttgacataccatctcatccctgcgtgtctc

SEQ ID NO: 6 - DNA, 45 bp, synthetic construct
  misc_feature 1..45: note = synthetic oligonucleotide
  source 1..45: mol_type = other DNA
caagcagaagacggcatacgagatgtgactggagttcagacgtgt

SEQ ID NO: 7 - DNA, 29 bp, synthetic construct
  misc_feature 1..29: note = synthetic oligonucleotide
  source 1..29: mol_type = other DNA
aatgatacggcgaccaccgagatctacac

SEQ ID NO: 8 - DNA, 24 bp, synthetic construct
  misc_feature 1..24: note = synthetic oligonucleotide
  source 1..24: mol_type = other DNA
caagcagaagacggcatacgagat

SEQ ID NO: 9 - DNA, 21 bp, synthetic construct
  misc_feature 1..21: note = synthetic oligonucleotide
  source 1..21: mol_type = other DNA
tctctggcctccacttttgct

SEQ ID NO: 10 - DNA, 21 bp, synthetic construct
  misc_feature 1..21: note = synthetic oligonucleotide
  source 1..21: mol_type = other DNA
gaggtggtatacagtgcccat

SEQ ID NO: 11 - DNA, 21 bp, synthetic construct
  misc_feature 1..21: note = synthetic oligonucleotide
  source 1..21: mol_type = other DNA
aggattgatggcagattcagt

SEQ ID NO: 12 - DNA, 24 bp, synthetic construct
  misc_feature 1..24: note = synthetic oligonucleotide
  source 1..24: mol_type = other DNA
gactattttaagtattgcgtctgt

SEQ ID NO: 13 - DNA, 21 bp, synthetic construct
  misc_feature 1..21: note = synthetic oligonucleotide
  source 1..21: mol_type = other DNA
cccttttctattgcactccac

SEQ ID NO: 14 - DNA, 22 bp, synthetic construct
  misc_feature 1..22: note = synthetic oligonucleotide
  source 1..22: mol_type = other DNA
atgaacagagaagtcatttgcc

SEQ ID NO: 15 - DNA, 22 bp, synthetic construct
  misc_feature 1..22: note = synthetic oligonucleotide
  source 1..22: mol_type = other DNA
gccagatgtcagtcttgttcac

SEQ ID NO: 16 - DNA, 20 bp, synthetic construct
  misc_feature 1..20: note = synthetic oligonucleotide
  source 1..20: mol_type = other DNA
gctaagccctttcctacagc

SEQ ID NO: 17 - DNA, 21 bp, synthetic construct
  misc_feature 1..21: note = synthetic oligonucleotide
  source 1..21: mol_type = other DNA
ttctcttagagtgaggctggg

SEQ ID NO: 18 - DNA, 22 bp, synthetic construct
  misc_feature 1..22: note = synthetic oligonucleotide
  source 1..22: mol_type = other DNA
tggagaacattccttagcaccc

SEQ ID NO: 19 - DNA, 21 bp, synthetic construct
  misc_feature 1..21: note = synthetic oligonucleotide
  source 1..21: mol_type = other DNA
cacagagtggctgaagaacca

SEQ ID NO: 20 - DNA, 21 bp, synthetic construct
  misc_feature 1..21: note = synthetic oligonucleotide
  source 1..21: mol_type = other DNA
ggctcagttgcataaaccgat

SEQ ID NO: 21 - DNA, 21 bp, synthetic construct
  misc_feature 1..21: note = synthetic oligonucleotide
  source 1..21: mol_type = other DNA
cgcagcccaagtcctaacaca

SEQ ID NO: 22 - DNA, 21 bp, synthetic construct
  misc_feature 1..21: note = synthetic oligonucleotide
  source 1..21: mol_type = other DNA
ttgttgtagggctggctctgt

SEQ ID NO: 23 - DNA, 19 bp, synthetic construct
  misc_feature 1..19: note = synthetic oligonucleotide
  source 1..19: mol_type = other DNA
gagagagcctgccacccat

SEQ ID NO: 24 - DNA, 21 bp, synthetic construct
  misc_feature 1..21: note = synthetic oligonucleotide
  source 1..21: mol_type = other DNA
tacaagggtgagaaaggaggc

SEQ ID NO: 25 - DNA, 23 bp, synthetic construct
  misc_feature 1..23: note = synthetic oligonucleotide
  source 1..23: mol_type = other DNA
ctatgcccctataagaccaccct

SEQ ID NO: 26 - DNA, 20 bp, synthetic construct
  misc_feature 1..20: note = synthetic oligonucleotide
  source 1..20: mol_type = other DNA
gcaggccaatggaacacctc

SEQ ID NO: 27 - DNA, 23 bp, synthetic construct
  misc_feature 1..23: note = synthetic oligonucleotide
  source 1..23: mol_type = other DNA
aatattctttgggaggacagtcg

SEQ ID NO: 28 - DNA, 23 bp, synthetic construct
  misc_feature 1..23: note = synthetic oligonucleotide
  source 1..23: mol_type = other DNA
tgcagtatgaatggagtaagtga

SEQ ID NO: 29 - DNA, 21 bp, synthetic construct
  misc_feature 1..21: note = synthetic oligonucleotide
  source 1..21: mol_type = other DNA
cctctagtctttggtctgcat

SEQ ID NO: 30 - DNA, 23 bp, synthetic construct
  misc_feature 1..23: note = synthetic oligonucleotide
  source 1..23: mol_type = other DNA
ctgactaattagccaagactgtg

SEQ ID NO: 31 - DNA, 21 bp, synthetic construct
  misc_feature 1..21: note = synthetic oligonucleotide
  source 1..21: mol_type = other DNA
tttaagctgtttccattgggg

SEQ ID NO: 32 - DNA, 20 bp, synthetic construct
  misc_feature 1..20: note = synthetic oligonucleotide
  source 1..20: mol_type = other DNA
agaattgtctgccctccaca

SEQ ID NO: 33 - DNA, 23 bp, synthetic construct
  misc_feature 1..23: note = synthetic oligonucleotide
  source 1..23: mol_type = other DNA
acgaagaggtcctgataagactg

SEQ ID NO: 34 - DNA, 21 bp, synthetic construct
  misc_feature 1..21: note = synthetic oligonucleotide
  source 1..21: mol_type = other DNA
tcctaagtgacgctaacctcc

SEQ ID NO: 35 - DNA, 23 bp, synthetic construct
  misc_feature 1..23: note = synthetic oligonucleotide
  source 1..23: mol_type = other DNA
gtcacaattttgaatccctgctg

SEQ ID NO: 36 - DNA, 20 bp, synthetic construct
  misc_feature 1..20: note = synthetic oligonucleotide
  source 1..20: mol_type = other DNA
tcatgtgctcactcctgctt

SEQ ID NO: 37 - DNA, 22 bp, synthetic construct
  misc_feature 1..22: note = synthetic oligonucleotide
  source 1..22: mol_type = other DNA
gtacgccgcagagtctagctca

SEQ ID NO: 38 - DNA, 22 bp, synthetic construct
  misc_feature 1..22: note = synthetic oligonucleotide
  source 1..22: mol_type = other DNA
aaactagagtcgctttggacag

SEQ ID NO: 39 - DNA, 23 bp, synthetic construct
  misc_feature 1..23: note = synthetic oligonucleotide
  source 1..23: mol_type = other DNA
tgatgaagacttgaaaagctcct

SEQ ID NO: 40 - DNA, 21 bp, synthetic construct
  misc_feature 1..21: note = synthetic oligonucleotide
  source 1..21: mol_type = other DNA
gcagccccaacaagactgaca

SEQ ID NO: 41 - DNA, 21 bp, synthetic construct
  misc_feature 1..21: note = synthetic oligonucleotide
  source 1..21: mol_type = other DNA
cctaccatgccaagtgtctgc

SEQ ID NO: 42 - DNA, 22 bp, synthetic construct
  misc_feature 1..22: note = synthetic oligonucleotide
  source 1..22: mol_type = other DNA
tcctgagacttttctgcctttc

SEQ ID NO: 43 - DNA, 21 bp, synthetic construct
  misc_feature 1..21: note = synthetic oligonucleotide
  source 1..21: mol_type = other DNA
cagtgagcacaggcagctggg

SEQ ID NO: 44 - DNA, 19 bp, synthetic construct
  misc_feature 1..19: note = synthetic oligonucleotide
  source 1..19: mol_type = other DNA
cctcggcaccataggggtc

SEQ ID NO: 45 - DNA, 22 bp, synthetic construct
  misc_feature 1..22: note = synthetic oligonucleotide
  source 1..22: mol_type = other DNA
gcagcactactgtgagttgctt

SEQ ID NO: 46 - DNA, 20 bp, synthetic construct
  misc_feature 1..20: note = synthetic oligonucleotide
  source 1..20: mol_type = other DNA
ggtcggggtggggagtccag

SEQ ID NO: 47 - DNA, 23 bp, synthetic construct
  misc_feature 1..23: note = synthetic oligonucleotide
  source 1..23: mol_type = other DNA
tgccaacttctgtctgggaccct

SEQ ID NO: 48 - DNA, 21 bp, synthetic construct
  misc_feature 1..21: note = synthetic oligonucleotide
  source 1..21: mol_type = other DNA
ctgtgctgggactcatttgct

SEQ ID NO: 49 - DNA, 21 bp, synthetic construct
  misc_feature 1..21: note = synthetic oligonucleotide
  source 1..21: mol_type = other DNA
gaggctggataagatctcagg

SEQ ID NO: 50 - DNA, 21 bp, synthetic construct
  misc_feature 1..21: note = synthetic oligonucleotide
  source 1..21: mol_type = other DNA
tttgaggggaatcttcagagc

SEQ ID NO: 51 - DNA, 22 bp, synthetic construct
  misc_feature 1..22: note = synthetic oligonucleotide
  source 1..22: mol_type = other DNA
tgccttggactcaggaagggaa

SEQ ID NO: 52 - DNA, 23 bp, synthetic construct
  misc_feature 1..23: note = synthetic oligonucleotide
  source 1..23: mol_type = other DNA
gagacatttgtgatgttggctgt

SEQ ID NO: 53 - DNA, 54 bp, synthetic construct
  misc_feature 1..54: note = synthetic oligonucleotide
  source 1..54: mol_type = other DNA
gtgactggagttcagacgtgtgctcttccgatctccccggtggtatgaaagctg

SEQ ID NO: 54 - DNA, 57 bp, synthetic construct
  misc_feature 1..57: note = synthetic oligonucleotide
  source 1..57: mol_type = other DNA
gtgactggagttcagacgtgtgctcttccgatcttgccttccaccagcctcacatca

SEQ ID NO: 55 - DNA, 60 bp, synthetic construct
  misc_feature 1..60: note = synthetic oligonucleotide
  source 1..60: mol_type = other DNA
gtgactggagttcagacgtgtgctcttccgatcttttcctttggagacaggggttctcta

SEQ ID NO: 56 - DNA, 56 bp, synthetic construct
  misc_feature 1..56: note = synthetic oligonucleotide
  source 1..56: mol_type = other DNA
gtgactggagttcagacgtgtgctcttccgatcttttgtctaaaatgcctccgtgt

SEQ ID NO: 57 - DNA, 58 bp, synthetic construct
  misc_feature 1..58: note = synthetic oligonucleotide
  source 1..58: mol_type = other DNA
gtgactggagttcagacgtgtgctcttccgatcttctctcattgaacctggagctctg

SEQ ID NO: 58 - DNA, 57 bp, synthetic construct
  misc_feature 1..57: note = synthetic oligonucleotide
  source 1..57: mol_type = other DNA
gtgactggagttcagacgtgtgctcttccgatctcaacaccacatccaaatacaggg

SEQ ID NO: 59 - DNA, 58 bp, synthetic construct
  misc_feature 1..58: note = synthetic oligonucleotide
  source 1..58: mol_type = other DNA
gtgactggagttcagacgtgtgctcttccgatcttccttcatccctgtacatgcctag

SEQ ID NO: 60 - DNA, 56 bp, synthetic construct
  misc_feature 1..56: note = synthetic oligonucleotide
  source 1..56: mol_type = other DNA
gtgactggagttcagacgtgtgctcttccgatctttttattcccttcccggcccat

SEQ ID NO: 61 - DNA, 55 bp, synthetic construct
  misc_feature 1..55: note = synthetic oligonucleotide
  source 1..55: mol_type = other DNA
gtgactggagttcagacgtgtgctcttccgatctgtgcagagcctgggaagtgga

SEQ ID NO: 62 - DNA, 58 bp, synthetic construct
  misc_feature 1..58: note = synthetic oligonucleotide
  source 1..58: mol_type = other DNA
gtgactggagttcagacgtgtgctcttccgatcttgtaaagaggcagactagacgtgg

SEQ ID NO: 63 - DNA, 54 bp, synthetic construct
  misc_feature 1..54: note = synthetic oligonucleotide
  source 1..54: mol_type = other DNA
gtgactggagttcagacgtgtgctcttccgatctgactgggccttggacagtgg

SEQ ID NO: 64 - DNA, 57 bp, synthetic construct
  misc_feature 1..57: note = synthetic oligonucleotide
  source 1..57: mol_type = other DNA
gtgactggagttcagacgtgtgctcttccgatctatggtgatggagtgtaaactggg

SEQ ID NO: 65 - DNA, 59 bp, synthetic construct
  misc_feature 1..59: note = synthetic oligonucleotide
  source 1..59: mol_type = other DNA
gtgactggagttcagacgtgtgctcttccgatctagtgcttgtcctccttgtagttggg

SEQ ID NO: 66 - DNA, 58 bp, synthetic construct
  misc_feature 1..58: note = synthetic oligonucleotide
  source 1..58: mol_type = other DNA
gtgactggagttcagacgtgtgctcttccgatctaaatttggtgctttggcgttgtaa

SEQ ID NO: 67 - DNA, 57 bp, synthetic construct
  misc_feature 1..57: note = synthetic oligonucleotide
  source 1..57: mol_type = other DNA
gtgactggagttcagacgtgtgctcttccgatctattgacattggcaactcctggtg

SEQ ID NO: 68 - DNA, 55 bp, synthetic construct
  misc_feature 1..55: note = synthetic oligonucleotide
  source 1..55: mol_type = other DNA
gtgactggagttcagacgtgtgctcttccgatctcagtgtctcattggcaccatc

SEQ ID NO: 69 - DNA, 57 bp, synthetic construct
  misc_feature 1..57: note = synthetic oligonucleotide
  source 1..57: mol_type = other DNA
gtgactggagttcagacgtgtgctcttccgatctcaacagtgcacctaaaggactca

SEQ ID NO: 70 - DNA, 58 bp, synthetic construct
  misc_feature 1..58: note = synthetic oligonucleotide
  source 1..58: mol_type = other DNA
gtgactggagttcagacgtgtgctcttccgatctaccatgctgtgacaacccaactga

SEQ ID NO: 71 - DNA, 55 bp, synthetic construct
  misc_feature 1..55: note = synthetic oligonucleotide
  source 1..55: mol_type = other DNA
gtgactggagttcagacgtgtgctcttccgatctgacctcagtttcatctggctt

SEQ ID NO: 72 - DNA, 56 bp, synthetic construct
  misc_feature 1..56: note = synthetic oligonucleotide
  source 1..56: mol_type = other DNA
gtgactggagttcagacgtgtgctcttccgatctatctgttcccattagcaggtga

SEQ ID NO: 73 - DNA, 61 bp, synthetic construct
  misc_feature 1..61: note = synthetic oligonucleotide
  source 1..61: mol_type = other DNA
gtgactggagttcagacgtgtgctcttccgatctatcttcccctggcttctaggatgtatg

SEQ ID NO: 74 - DNA, 55 bp, synthetic construct
  misc_feature 1..55: note = synthetic oligonucleotide
  source 1..55: mol_type = other DNA
gtgactggagttcagacgtgtgctcttccgatctgattgcggggttgtatctggg

SEQ ID NO: 75 - DNA, 57 bp, synthetic construct
  misc_feature 1..57: note = synthetic oligonucleotide
  source 1..57: mol_type = other DNA
gtgactggagttcagacgtgtgctcttccgatctttatatgatgggaggggttcttc

SEQ ID NO: 76 - DNA, 55 bp, synthetic construct
  misc_feature 1..55: note = synthetic oligonucleotide
  source 1..55: mol_type = other DNA
gtgactggagttcagacgtgtgctcttccgatctgaaggtgtaaaggggtcccaa

SEQ ID NO: 77 - DNA, 55 bp, synthetic construct
  misc_feature 1..55: note = synthetic oligonucleotide
  source 1..55: mol_type = other DNA
gtgactggagttcagacgtgtgctcttccgatctctcgtagaaggaggggttggg

SEQ ID NO: 78 - DNA, 55 bp, synthetic construct
  misc_feature 1..55: note = synthetic oligonucleotide
  source 1..55: mol_type = other DNA
gtgactggagttcagacgtgtgctcttccgatctccaatgctcactgccttccct

SEQ ID NO: 79 - DNA, 55 bp, synthetic construct
  misc_feature 1..55: note = synthetic oligonucleotide
  source 1..55: mol_type = other DNA
gtgactggagttcagacgtgtgctcttccgatctgatactgtggttgggtgcctt

SEQ ID NO: 80 - DNA, 55 bp, synthetic construct
  misc_feature 1..55: note = synthetic oligonucleotide
  source 1..55: mol_type = other DNA
gtgactggagttcagacgtgtgctcttccgatctcttgtgcctgagctgtaggga

SEQ ID NO: 81 - DNA, 56 bp, synthetic construct
  misc_feature 1..56: note = synthetic oligonucleotide
  source 1..56: mol_type = other DNA
gtgactggagttcagacgtgtgctcttccgatctaccttaaaggaggccatctcgt

SEQ ID NO: 82 - DNA, 55 bp, synthetic construct
  misc_feature 1..55: note = synthetic oligonucleotide
  source 1..55: mol_type = other DNA
gtgactggagttcagacgtgtgctcttccgatctacctaagccaagggtaactcg

SEQ ID NO: 83 - DNA, 55 bp, synthetic construct
  misc_feature 1..55: note = synthetic oligonucleotide
  source 1..55: mol_type = other DNA
gtgactggagttcagacgtgtgctcttccgatctccgtgagcgtatctgctgtcc

SEQ ID NO: 84 - DNA, 60 bp, synthetic construct
  misc_feature 1..60: note = synthetic oligonucleotide
  source 1..60: mol_type = other DNA
gtgactggagttcagacgtgtgctcttccgatctccaaagcatgacctgacattgacacc

SEQ ID NO: 85 - DNA, 55 bp, synthetic construct
  misc_feature 1..55: note = synthetic oligonucleotide
  source 1..55: mol_type = other DNA
gtgactggagttcagacgtgtgctcttccgatctcgcagtggggctgtgtggtaa

SEQ ID NO: 86 - DNA, 55 bp, synthetic construct
  misc_feature 1..55: note = synthetic oligonucleotide
  source 1..55: mol_type = other DNA
gtgactggagttcagacgtgtgctcttccgatctcctctgcctgttttctgggac

SEQ ID NO: 87 - DNA, 59 bp, synthetic construct
  misc_feature 1..59: note = synthetic oligonucleotide
  source 1..59: mol_type = other DNA
gtgactggagttcagacgtgtgctcttccgatctaaagggtccttatttgcaaggctac

SEQ ID NO: 88 - DNA, 56 bp, synthetic construct
  misc_feature 1..56: note = synthetic oligonucleotide
  source 1..56: mol_type = other DNA
gtgactggagttcagacgtgtgctcttccgatctttaggattcgcccattcctgtc

SEQ ID NO: 89 - DNA, 57 bp, synthetic construct
  misc_feature 1..57: note = synthetic oligonucleotide
  source 1..57: mol_type = other DNA
gtgactggagttcagacgtgtgctcttccgatctcttgctctgtgctgctacttggg

SEQ ID NO: 90 - DNA, 60 bp, synthetic construct
  misc_feature 1..60: note = synthetic oligonucleotide
  source 1..60: mol_type = other DNA
gtgactggagttcagacgtgtgctcttccgatctagccaaacagagaagactcaggtgac

SEQ ID NO: 91 - DNA, 57 bp, synthetic construct
  misc_feature 1..57: note = synthetic oligonucleotide
  source 1..57: mol_type = other DNA
gtgactggagttcagacgtgtgctcttccgatctggaccctgcccctatatttggag

SEQ ID NO: 92 - DNA, 56 bp, synthetic construct
  misc_feature 1..56: note = synthetic oligonucleotide
  source 1..56: mol_type = other DNA
gtgactggagttcagacgtgtgctcttccgatctctatagaaagtggccttgggag

SEQ ID NO: 93 - DNA, 56 bp, synthetic construct
  misc_feature 1..56: note = synthetic oligonucleotide
  source 1..56: mol_type = other DNA
gtgactggagttcagacgtgtgctcttccgatctgcaatgcacagccttcctcaca

SEQ ID NO: 94 - DNA, 55 bp, synthetic construct
  misc_feature 1..55: note = synthetic oligonucleotide
  source 1..55: mol_type = other DNA
gtgactggagttcagacgtgtgctcttccgatctgcctgcttctcctgtttcctc

SEQ ID NO: 95 - DNA, 59 bp, synthetic construct
  misc_feature 1..59: note = synthetic oligonucleotide
  source 1..59: mol_type = other DNA
gtgactggagttcagacgtgtgctcttccgatctcttcccaaaagatttccacgtgtgt

SEQ ID NO: 96 - DNA, 57 bp, synthetic construct
  misc_feature 1..57: note = synthetic oligonucleotide
  source 1..57: mol_type = other DNA
gtgactggagttcagacgtgtgctcttccgatctaatctttgttaccttcgctgtga